European Patent Application EP 4 674 955 A1, published January 7, 2026. Title: 具有聚酯降解活性的酯酶突变体及其应用. Applicant: 天津大学. The sequence listing filed with the application follows.

SEQUENCE LISTING (124 sequences)

SEQ ID NO: 1 - protein, 263 aa, synthetic construct
QTNPYARGPNPTAASLEASAGPFTVRSFTVSRPSGYGAGTVYYPTNAGGTVGAIAIVPGYTARQSSIKWWGPRLASHGFVVITIDTNSTLDQPSSRSSQQMAALRQVASLNGTSSSPIYGKVDTARMGVMGWSMGGGGSLISAANNPSLKAAAPQAPWDSSTNFSSVTVPTLIFACENDSIAPVNSSALPIYDSMSRNAKQFLEINGGSHSCANSGNSNQALIGKKGVAWMKRFMDNDTRYSTFACENPNSTRVSDFRTANCS

SEQ ID NO: 2 - DNA, 789 bp, synthetic construct
  source 1..789: mol_type = other DNA
caaaccaatccttatgcccgtggtcctaatcctaccgccgcgagcttagaagcaagcgccggtccttttaccgttcgtagctttaccgttagccgcccatcaggttatggtgccggtaccgtttactatccaaccaacgccggtggtaccgttggtgccattgccattgttccaggttacaccgcccgtcaaagcagcattaagtggtggggtccgcgtttggccagccatggttttgttgttatcaccatcgataccaacagcaccttggatcaaccaagcagccgtagcagccaacaaatggccgccttgcgtcaagttgccagcctgaacggtactagcagcagcccaatttacggtaaggttgataccgcccgtatgggtgttatgggttggagcatgggtggtggcggtagcttgattagcgccgccaacaacccaagcttgaaagccgcagcaccacaagccccatgggatagcagcaccaactttagcagcgttaccgttcctaccttgatttttgcctgtgagaacgatagcattgccccagttaacagcagcgccttgccaatttacgatagcatgagccgtaacgccaagcaattcttagaaatcaacggtggtagccatagctgtgccaacagcggtaacagcaaccaagccttgattggtaagaaaggcgttgcctggatgaagcgttttatggataacgatacccgttacagcacctttgcctgtgaaaacccaaacagcacccgtgttagcgattttcgtaccgccaactgtagc

SEQ ID NO: 3 - protein, 263 aa, synthetic construct
QTNPYARGPNPTAASLEASAGPFTVRSFTVSRPSGYGAGTVYYPTNAGGTVGAIAIVPGYTARQSSIKWWGPRLASHGFVVITIDTNSTLDQPESRSSQQMAALRQVASLNGTSSSPIYGKVDTARMGVMGWSMGGGGSLISAANNPSLKAAAPQAPWHSSTNFSSVTVPTLIFACENDSIAPVNSSALPIYDSMSRNAKQFLEICGGSHSCANTGNSDQALIGKKGVAWMKRFMDNDTRYSTFACENPNSTRVCDFRTANCS

SEQ ID NO: 4 - DNA, 789 bp, synthetic construct
  source 1..789: mol_type = other DNA
cagaccaatccgtatgcccgcggcccgaatccgaccgcggcgtcattagaagcgagcgcgggtccttttaccgttcgctcatttaccgttagccgcccgagcggctatggcgcgggcactgtttattatccgaccaacgcgggcggcaccgtgggcgcgattgcgattgttcctggctataccgcgcgtcagagcagcattaaatggtggggcccgcgcctggcgagccacggttttgttgttattaccattgataccaacagcaccctggatcagccggaaagccgcagcagccagcaaatggcggcgttacgtcaagtggcgagcctgaacggtaccagcagcagccctatttatggcaaagtggataccgcgcgtatgggcgtgatgggctggtcaatgggtggtggcggtagcttaattagcgcggcgaataatccgagcctgaaagcggcggcgccgcaggcgccttggcatagcagcaccaattttagcagcgtgaccgtgccgaccctgatttttgcgtgcgaaaacgatagcattgcgccggtgaacagcagcgcgttacctatttatgatagcatgagccgcaacgcgaaacagtttctggaaatttgcggcggcagccatagctgcgcgaacaccggtaatagcgatcaggcgttaattggcaaaaagggcgtggcgtggatgaaacgctttatggataacgatacccgctatagcacctttgcgtgcgaaaacccgaacagcacccgcgtgtgtgattttcgcaccgcgaactgcagc

SEQ ID NO: 5 - DNA, 32 bp, synthetic construct
  source 1..32: mol_type = other DNA
tgcgtgccagaacgatagcattgcgccggtga

SEQ ID NO: 6 - DNA, 32 bp, synthetic construct
  source 1..32: mol_type = other DNA
tatcgttctggcacgcaaaaatcagggtcggc

SEQ ID NO: 7 - DNA, 28 bp, synthetic construct
  source 1..28: mol_type = other DNA
tgcgtgccagaacgatagcattgcgccg

SEQ ID NO: 8 - DNA, 30 bp, synthetic construct
  source 1..30: mol_type = other DNA
tatcgttctggcacgcaaaaatcagggtcg

SEQ ID NO: 9 - DNA, 33 bp, synthetic construct
  source 1..33: mol_type = other DNA
aaatttgcggcgcgagccatagctgcgcgaaca

SEQ ID NO: 10 - DNA, 27 bp, synthetic construct
  source 1..27: mol_type = other DNA
gctcgcgccgcaaatttccagaaactg

SEQ ID NO: 11 - DNA, 32 bp, synthetic construct
  source 1..32: mol_type = other DNA
tgcgaagccgatagcattgcgccggtgaacag

SEQ ID NO: 12 - DNA, 32 bp, synthetic construct
  source 1..32: mol_type = other DNA
atgctatcggcttcgcacgcaaaaatcagggt

SEQ ID NO: 13 - DNA, 32 bp, synthetic construct
  source 1..32: mol_type = other DNA
aaacgatacgattgcgccggtgaacagcagcg

SEQ ID NO: 14 - DNA, 32 bp, synthetic construct
  source 1..32: mol_type = other DNA
gcgcaattgcatcgttttcgcacgcaaaaatc

SEQ ID NO: 15 - DNA, 32 bp, synthetic construct
  source 1..32: mol_type = other DNA
aaacgatctgattgcgccggtgaacagcagcg

SEQ ID NO: 16 - DNA, 32 bp, synthetic construct
  source 1..32: mol_type = other DNA
gcgcaatcagatcgttttcgcacgcaaaaatc

SEQ ID NO: 17 - DNA, 32 bp, synthetic construct
  source 1..32: mol_type = other DNA
aaacgatgtgattgcgccggtgaacagcagcg

SEQ ID NO: 18 - DNA, 32 bp, synthetic construct
  source 1..32: mol_type = other DNA
gcgcaatcacatcgttttcgcacgcaaaaatc

SEQ ID NO: 19 - DNA, 32 bp, synthetic construct
  source 1..32: mol_type = other DNA
aaacgattcggttgcgccggtgaacagcagcg

SEQ ID NO: 20 - DNA, 32 bp, synthetic construct
  source 1..32: mol_type = other DNA
gcgcaaccgaatcgttttcgcacgcaaaaatc

SEQ ID NO: 21 - DNA, 33 bp, synthetic construct; identical to SEQ ID NO: 9
  source 1..33: mol_type = other DNA

SEQ ID NO: 22 - DNA, 32 bp, synthetic construct
  source 1..32: mol_type = other DNA
gctcgcgccgcaaatttccagaaactgtttcg

SEQ ID NO: 23 - DNA, 36 bp, synthetic construct
  source 1..36: mol_type = other DNA
aaatttgcggcggcacccatagctgcgcgaacaccg

SEQ ID NO: 24 - DNA, 32 bp, synthetic construct
  source 1..32: mol_type = other DNA
ggtgccgccgcaaatttccagaaactgtttcg

SEQ ID NO: 25 - DNA, 32 bp, synthetic construct
  source 1..32: mol_type = other DNA
cagccattattgcgcgaacaccggtaatagcg

SEQ ID NO: 26 - DNA, 32 bp, synthetic construct
  source 1..32: mol_type = other DNA
tcgcgcaataatggctgccgccgcaaatttcc

SEQ ID NO: 27 - DNA, 35 bp, synthetic construct
  source 1..35: mol_type = other DNA
cgtgccaaaacgatctgattgcgccggtgaacagc

SEQ ID NO: 28 - DNA, 33 bp, synthetic construct
  source 1..33: mol_type = other DNA
tcagatcgttttggcacgcaaaaatcagggtcg

SEQ ID NO: 29 - DNA, 34 bp, synthetic construct
  source 1..34: mol_type = other DNA
ccagaacgatagcgtggcgccggtgaacagcagc

SEQ ID NO: 30 - DNA, 36 bp, synthetic construct
  source 1..36: mol_type = other DNA
ccacgctatcgttctggcacgcaaaaatcagggtcg

SEQ ID NO: 31 - DNA, 27 bp, synthetic construct
  source 1..27: mol_type = other DNA
tgccaggcggatagcattgcgccggtg

SEQ ID NO: 32 - DNA, 35 bp, synthetic construct
  source 1..35: mol_type = other DNA
aatgctatccgcctggcacgcaaaaatcagggtcg

SEQ ID NO: 33 - DNA, 31 bp, synthetic construct
  source 1..31: mol_type = other DNA
cgaagcggatctgattgcgccggtgaacagc

SEQ ID NO: 34 - DNA, 32 bp, synthetic construct
  source 1..32: mol_type = other DNA
caatcagatccgcttcgcacgcaaaaatcagg

SEQ ID NO: 35 - DNA, 36 bp, synthetic construct
  source 1..36: mol_type = other DNA
tgcgaagcggatagcgtggcgccggtgaacagcagc

SEQ ID NO: 36 - DNA, 31 bp, synthetic construct
  source 1..31: mol_type = other DNA
cacgctatccgcttcgcacgcaaaaatcagg

SEQ ID NO: 37 - DNA, 34 bp, synthetic construct
  source 1..34: mol_type = other DNA
gtgccagaacgataccattgcgccggtgaacagc

SEQ ID NO: 38 - DNA, 34 bp, synthetic construct
  source 1..34: mol_type = other DNA
atggtatcgttctggcacgcaaaaatcagggtcg

SEQ ID NO: 39 - DNA, 31 bp, synthetic construct
  source 1..31: mol_type = other DNA
cgaagccgataccattgcgccggtgaacagc

SEQ ID NO: 40 - DNA, 32 bp, synthetic construct
  source 1..32: mol_type = other DNA
caatggtatcggcttcgcacgcaaaaatcagg

SEQ ID NO: 41 - DNA, 36 bp, synthetic construct
  source 1..36: mol_type = other DNA
tgcgaaaacgataccgtggcgccggtgaacagcagc

SEQ ID NO: 42 - DNA, 25 bp, synthetic construct
  source 1..25: mol_type = other DNA
cacggtatcgttttcgcacgcaaaa

SEQ ID NO: 43 - DNA, 36 bp, synthetic construct
  source 1..36: mol_type = other DNA
tgcgaaaacgatctggtggcgccggtgaacagcagc

SEQ ID NO: 44 - DNA, 25 bp, synthetic construct
  source 1..25: mol_type = other DNA
caccagatcgttttcgcacgcaaaa

SEQ ID NO: 45 - DNA, 34 bp, synthetic construct
  source 1..34: mol_type = other DNA
gtgccagaacgatgtgattgcgccggtgaacagc

SEQ ID NO: 46 - DNA, 34 bp, synthetic construct
  source 1..34: mol_type = other DNA
atcacatcgttctggcacgcaaaaatcagggtcg

SEQ ID NO: 47 - DNA, 31 bp, synthetic construct
  source 1..31: mol_type = other DNA
cgaagcggatgtgattgcgccggtgaacagc

SEQ ID NO: 48 - DNA, 32 bp, synthetic construct
  source 1..32: mol_type = other DNA
caatcacatccgcttcgcacgcaaaaatcagg

SEQ ID NO: 49 - DNA, 36 bp, synthetic construct
  source 1..36: mol_type = other DNA
tgcgaaaacgatgtggtggcgccggtgaacagcagc

SEQ ID NO: 50 - DNA, 25 bp, synthetic construct
  source 1..25: mol_type = other DNA
caccacatcgttttcgcacgcaaaa

SEQ ID NO: 51 - DNA, 33 bp, synthetic construct
  source 1..33: mol_type = other DNA
aaatttgcggcgcgacccatagctgcgcgaaca

SEQ ID NO: 52 - DNA, 32 bp, synthetic construct
  source 1..32: mol_type = other DNA
ggtcgcgccgcaaatttccagaaactgtttcg

SEQ ID NO: 53 - DNA, 32 bp, synthetic construct
  source 1..32: mol_type = other DNA
cggcgcgagccattattgcgcgaacaccggta

SEQ ID NO: 54 - DNA, 34 bp, synthetic construct
  source 1..34: mol_type = other DNA
aataatggctcgcgccgcaaatttccagaaactg

SEQ ID NO: 55 - DNA, 32 bp, synthetic construct
  source 1..32: mol_type = other DNA
cacccattattgcgcgaacaccggtaatagcg

SEQ ID NO: 56 - DNA, 34 bp, synthetic construct
  source 1..34: mol_type = other DNA
tcgcgcaataatgggtgccgccgcaaatttccag

SEQ ID NO: 57 - DNA, 27 bp, synthetic construct
  source 1..27: mol_type = other DNA
tgcgaagcggatagcattgcgccggtg

SEQ ID NO: 58 - DNA, 30 bp, synthetic construct
  source 1..30: mol_type = other DNA
atgctatccgcttcgcacgcaaaaatcagg

SEQ ID NO: 59 - DNA, 33 bp, synthetic construct; identical to SEQ ID NO: 9
  source 1..33: mol_type = other DNA

SEQ ID NO: 60 - DNA, 27 bp, synthetic construct
  source 1..27: mol_type = other DNA
gctcgcgccgcaaatttccagaaactg

SEQ ID NO: 61 - DNA, 27 bp, synthetic construct
  source 1..27: mol_type = other DNA
tgcgaagcggatagcattgcgccggtg

SEQ ID NO: 62 - DNA, 30 bp, synthetic construct; identical to SEQ ID NO: 58
  source 1..30: mol_type = other DNA

SEQ ID NO: 63 - DNA, 36 bp, synthetic construct; identical to SEQ ID NO: 23
  source 1..36: mol_type = other DNA

SEQ ID NO: 64 - DNA, 21 bp, synthetic construct
  source 1..21: mol_type = other DNA
ggtgccgccgcaaatttccag

SEQ ID NO: 65 - DNA, 28 bp, synthetic construct
  source 1..28: mol_type = other DNA
aaacgataccattgcgccggtgaacagc

SEQ ID NO: 66 - DNA, 29 bp, synthetic construct
  source 1..29: mol_type = other DNA
gcgcaatggtatcgttttcgcacgcaaaa

SEQ ID NO: 67 - DNA, 33 bp, synthetic construct; identical to SEQ ID NO: 9
  source 1..33: mol_type = other DNA

SEQ ID NO: 68 - DNA, 27 bp, synthetic construct
  source 1..27: mol_type = other DNA
gctcgcgccgcaaatttccagaaactg

SEQ ID NO: 69 - DNA, 28 bp, synthetic construct
  source 1..28: mol_type = other DNA
aaacgataccattgcgccggtgaacagc

SEQ ID NO: 70 - DNA, 29 bp, synthetic construct
  source 1..29: mol_type = other DNA
gcgcaatggtatcgttttcgcacgcaaaa

SEQ ID NO: 71 - DNA, 36 bp, synthetic construct; identical to SEQ ID NO: 23
  source 1..36: mol_type = other DNA

SEQ ID NO: 72 - DNA, 21 bp, synthetic construct
  source 1..21: mol_type = other DNA
ggtgccgccgcaaatttccag

SEQ ID NO: 73 - DNA, 28 bp, synthetic construct
  source 1..28: mol_type = other DNA
aaacgataccattgcgccggtgaacagc

SEQ ID NO: 74 - DNA, 29 bp, synthetic construct
  source 1..29: mol_type = other DNA
gcgcaatggtatcgttttcgcacgcaaaa

SEQ ID NO: 75 - DNA, 28 bp, synthetic construct
  source 1..28: mol_type = other DNA
cagccattattgcgcgaacaccggtaat

SEQ ID NO: 76 - DNA, 28 bp, synthetic construct
  source 1..28: mol_type = other DNA
tcgcgcaataatggctgccgccgcaaat

SEQ ID NO: 77 - DNA, 28 bp, synthetic construct
  source 1..28: mol_type = other DNA
aaacgatctgattgcgccggtgaacagc

SEQ ID NO: 78 - DNA, 29 bp, synthetic construct
  source 1..29: mol_type = other DNA
gcgcaatcagatcgttttcgcacgcaaaa

SEQ ID NO: 79 - DNA, 33 bp, synthetic construct; identical to SEQ ID NO: 9
  source 1..33: mol_type = other DNA

SEQ ID NO: 80 - DNA, 27 bp, synthetic construct
  source 1..27: mol_type = other DNA
gctcgcgccgcaaatttccagaaactg

SEQ ID NO: 81 - DNA, 28 bp, synthetic construct
  source 1..28: mol_type = other DNA
aaacgatgtgattgcgccggtgaacagc

SEQ ID NO: 82 - DNA, 29 bp, synthetic construct
  source 1..29: mol_type = other DNA
gcgcaatcacatcgttttcgcacgcaaaa

SEQ ID NO: 83 - DNA, 33 bp, synthetic construct; identical to SEQ ID NO: 9
  source 1..33: mol_type = other DNA

SEQ ID NO: 84 - DNA, 27 bp, synthetic construct
  source 1..27: mol_type = other DNA
gctcgcgccgcaaatttccagaaactg

SEQ ID NO: 85 - DNA, 28 bp, synthetic construct
  source 1..28: mol_type = other DNA
aaacgatgtgattgcgccggtgaacagc

SEQ ID NO: 86 - DNA, 29 bp, synthetic construct
  source 1..29: mol_type = other DNA
gcgcaatcacatcgttttcgcacgcaaaa

SEQ ID NO: 87 - DNA, 36 bp, synthetic construct; identical to SEQ ID NO: 23
  source 1..36: mol_type = other DNA

SEQ ID NO: 88 - DNA, 32 bp, synthetic construct; identical to SEQ ID NO: 24
  source 1..32: mol_type = other DNA

SEQ ID NO: 89 - DNA, 32 bp, synthetic construct
  source 1..32: mol_type = other DNA
aaaacgatagcgtggcgccggtgaacagcagc

SEQ ID NO: 90 - DNA, 25 bp, synthetic construct
  source 1..25: mol_type = other DNA
cgccacgctatcgttttcgcacgca

SEQ ID NO: 91 - DNA, 33 bp, synthetic construct; identical to SEQ ID NO: 9
  source 1..33: mol_type = other DNA

SEQ ID NO: 92 - DNA, 32 bp, synthetic construct; identical to SEQ ID NO: 22
  source 1..32: mol_type = other DNA

SEQ ID NO: 93 - DNA, 28 bp, synthetic construct
  source 1..28: mol_type = other DNA
tgcgtgccagaacgatagcattgcgccg

SEQ ID NO: 94 - DNA, 30 bp, synthetic construct; identical to SEQ ID NO: 8
  source 1..30: mol_type = other DNA

SEQ ID NO: 95 - DNA, 36 bp, synthetic construct; identical to SEQ ID NO: 23
  source 1..36: mol_type = other DNA

SEQ ID NO: 96 - DNA, 21 bp, synthetic construct
  source 1..21: mol_type = other DNA
ggtgccgccgcaaatttccag

SEQ ID NO: 97 - DNA, 32 bp, synthetic construct; identical to SEQ ID NO: 15
  source 1..32: mol_type = other DNA

SEQ ID NO: 98 - DNA, 32 bp, synthetic construct; identical to SEQ ID NO: 16
  source 1..32: mol_type = other DNA

SEQ ID NO: 99 - DNA, 36 bp, synthetic construct; identical to SEQ ID NO: 23
  source 1..36: mol_type = other DNA

SEQ ID NO: 100 - DNA, 21 bp, synthetic construct
  source 1..21: mol_type = other DNA
ggtgccgccgcaaatttccag

SEQ ID NO: 101 - DNA, 32 bp, synthetic construct; identical to SEQ ID NO: 89
  source 1..32: mol_type = other DNA

SEQ ID NO: 102 - DNA, 32 bp, synthetic construct
  source 1..32: mol_type = other DNA
cgccacgctatcgttttcgcacgcaaaaatca

SEQ ID NO: 103 - DNA, 36 bp, synthetic construct; identical to SEQ ID NO: 23
  source 1..36: mol_type = other DNA

SEQ ID NO: 104 - DNA, 21 bp, synthetic construct
  source 1..21: mol_type = other DNA
ggtgccgccgcaaatttccag

SEQ ID NO: 105 - DNA, 32 bp, synthetic construct; identical to SEQ ID NO: 5
  source 1..32: mol_type = other DNA

SEQ ID NO: 106 - DNA, 32 bp, synthetic construct; identical to SEQ ID NO: 6
  source 1..32: mol_type = other DNA

SEQ ID NO: 107 - DNA, 28 bp, synthetic construct
  source 1..28: mol_type = other DNA
cagccattattgcgcgaacaccggtaat

SEQ ID NO: 108 - DNA, 28 bp, synthetic construct
  source 1..28: mol_type = other DNA
tcgcgcaataatggctgccgccgcaaat

SEQ ID NO: 109 - DNA, 32 bp, synthetic construct; identical to SEQ ID NO: 11
  source 1..32: mol_type = other DNA

SEQ ID NO: 110 - DNA, 32 bp, synthetic construct; identical to SEQ ID NO: 12
  source 1..32: mol_type = other DNA

SEQ ID NO: 111 - DNA, 28 bp, synthetic construct
  source 1..28: mol_type = other DNA
cagccattattgcgcgaacaccggtaat

SEQ ID NO: 112 - DNA, 28 bp, synthetic construct
  source 1..28: mol_type = other DNA
tcgcgcaataatggctgccgccgcaaat

SEQ ID NO: 113 - DNA, 32 bp, synthetic construct; identical to SEQ ID NO: 15
  source 1..32: mol_type = other DNA

SEQ ID NO: 114 - DNA, 32 bp, synthetic construct; identical to SEQ ID NO: 16
  source 1..32: mol_type = other DNA

SEQ ID NO: 115 - DNA, 28 bp, synthetic construct
  source 1..28: mol_type = other DNA
cagccattattgcgcgaacaccggtaat

SEQ ID NO: 116 - DNA, 28 bp, synthetic construct
  source 1..28: mol_type = other DNA
tcgcgcaataatggctgccgccgcaaat

SEQ ID NO: 117 - DNA, 32 bp, synthetic construct; identical to SEQ ID NO: 17
  source 1..32: mol_type = other DNA

SEQ ID NO: 118 - DNA, 32 bp, synthetic construct; identical to SEQ ID NO: 18
  source 1..32: mol_type = other DNA

SEQ ID NO: 119 - DNA, 28 bp, synthetic construct
  source 1..28: mol_type = other DNA
cagccattattgcgcgaacaccggtaat

SEQ ID NO: 120 - DNA, 28 bp, synthetic construct
  source 1..28: mol_type = other DNA
tcgcgcaataatggctgccgccgcaaat

SEQ ID NO: 121 - DNA, 32 bp, synthetic construct; identical to SEQ ID NO: 89
  source 1..32: mol_type = other DNA

SEQ ID NO: 122 - DNA, 32 bp, synthetic construct; identical to SEQ ID NO: 102
  source 1..32: mol_type = other DNA

SEQ ID NO: 123 - DNA, 28 bp, synthetic construct
  source 1..28: mol_type = other DNA
cagccattattgcgcgaacaccggtaat

SEQ ID NO: 124 - DNA, 28 bp, synthetic construct
  source 1..28: mol_type = other DNA
tcgcgcaataatggctgccgccgcaaat